European Patent Specification EP 3 628 337 B1, published May 28, 2025. Title: STERILIZATION AND FILTRATION OF PEPTIDE COMPOSITIONS. Applicant: 3-D Matrix, Ltd. The sequence listing filed with the application follows.

SEQUENCE LISTING (3 sequences)

SEQ ID NO: 1 - protein, 16 aa, Artificial Sequence
  synthetic
RADARADARADARADA

SEQ ID NO: 2 - protein, 12 aa, Artificial Sequence
  synthetic
KLDLKLDLKLDL

SEQ ID NO: 3 - protein, 13 aa, Artificial Sequence
  synthetic
IEIKIEIKIEIKI